European Patent Application EP 4 285 919 A1, published December 6, 2023. Title: Compositions and methods for inhibiting the activity of LAR family phosphatases. Applicant: CASE WESTERN RESERVE UNIVERSITY. Application EP. The sequence listing filed with the application follows.

SEQUENCE LISTING (93 sequences)

SEQ ID NO: 1 - protein, 33 aa, Mouse
PIPITDLADNIERLKANDGKLFSQEYESIDPGQ

SEQ ID NO: 2 - protein, 33 aa, Rat coronavirus; identical to SEQ ID NO: 1

SEQ ID NO: 3 - protein, 33 aa, Homo sapiens; identical to SEQ ID NO: 1

SEQ ID NO: 4 - protein, 33 aa, Mouse
PIPITDMAEHMERLKANDSLKLSQEYESIDPGQ

SEQ ID NO: 5 - protein, 33 aa, Rat coronavirus; identical to SEQ ID NO: 4

SEQ ID NO: 6 - protein, 33 aa, Homo sapiens
PIPIADMAEHTERLKANDSLKLSQEYESIDPGQ

SEQ ID NO: 7 - protein, 33 aa, Mouse
PIPILELADHIERLKANDNLKFSQEYESIDPGQ

SEQ ID NO: 8 - protein, 33 aa, Homo sapiens; identical to SEQ ID NO: 7

SEQ ID NO: 9 - protein, 22 aa, Xenopus borealis (PTP sigma)
DLAEHTEHLKANDNLKSQEYES

SEQ ID NO: 10 - protein, 22 aa, Green anole (PTP Sigma)
DHTEHELKANDNLKLSQEYESI

SEQ ID NO: 11 - protein, 24 aa, Zebrafish (PTP Sigma)
ELAEHTELLKANDNLKLSQEYESI

SEQ ID NO: 12 - protein, 24 aa, Talapia (PTP sigma)
ELAEHTELLKANDNLKLSQEYESI

SEQ ID NO: 13 - protein, 24 aa, Chicken (PTP Sigma)
ELAEHTEHLKANDNLKLSQEYESI

SEQ ID NO: 14 - protein, 24 aa, Fringilla coelebs
ELAEHTEHLKANDNLKLSQEYESI

SEQ ID NO: 15 - protein, 24 aa, Ornithorhynchus anatinus
ELAEHTDHLKANDNLKLSQEYESI

SEQ ID NO: 16 - protein, 24 aa, Sarcophilus harrisii
EMAEHTEHLKANDNLKLSQEYESI

SEQ ID NO: 17 - protein, 24 aa, Mustela putorius
DMAEHTERLKANDSLKLSQEYESI

SEQ ID NO: 18 - protein, 24 aa, Galago alleni
DMAEHTERLKANDSLKLSQEYESI

SEQ ID NO: 19 - protein, 24 aa, Callithrix aurita
DMAEHTERLKANDSLKLSQEYESI

SEQ ID NO: 20 - protein, 24 aa, Rattus rattus
DMAEHMERLKANDSLKLSQEYESI

SEQ ID NO: 21 - protein, 24 aa, Mus musculus
DMAEHMERLKANDSLKLSQEYESI

SEQ ID NO: 22 - protein, 24 aa, Canis familiaris
DMAEHTERLKANDSLKLSQEYESI

SEQ ID NO: 23 - protein, 24 aa, Sus barbatus
DMAEHTERLKANDSLKLSQEYESI

SEQ ID NO: 24 - protein, 24 aa, Bos primigenius
DMAEHTERLKANDSLKLSQEYESI

SEQ ID NO: 25 - protein, 24 aa, Ovis aries
DMAEHTERLKANDSLKLSQEYESI

SEQ ID NO: 26 - protein, 24 aa, Orcinus orca
DMAEHTERLKANDSLKLSQEYESI

SEQ ID NO: 27 - protein, 24 aa, Saimiri sciureus
DMAEHTERLKANDSLKLSQEYESI

SEQ ID NO: 28 - protein, 24 aa, Papio hamadryas
DMAEHTERLKANDSLKLSQEYESI

SEQ ID NO: 29 - protein, 24 aa, Primate calicivirus
DMAEHTERLKANDSLKLSQEYESI

SEQ ID NO: 30 - protein, 24 aa, Primate calicivirus
DMAEHTERLKANDSLKLSQEYESI

SEQ ID NO: 31 - protein, 24 aa, Macaca radiata
DMAEHTERLKANDSLKLSQEYESI

SEQ ID NO: 32 - protein, 24 aa, Pan troglodytes
DMAEHTERLKANDSLKLSQEYESI

SEQ ID NO: 33 - protein, 24 aa, Homo sapiens
DMAEHTERLKANDSLKLSQEYESI

SEQ ID NO: 34 - protein, 24 aa, Rat Lar
DLADNIERLKANDGLKFSQEYESI

SEQ ID NO: 35 - protein, 24 aa, RAT PTP Delta
ELADHIERLKANDNLKFSQEYESI

SEQ ID NO: 36 - protein, 24 aa, RAT PTP Alpha
KLEEEINRRMADDNKIFREEFNAL

SEQ ID NO: 37 - protein, 14 aa, synthetic construct
  VARIANT 3: note = X is T or M
EHXERLKANDSLKL

SEQ ID NO: 38 - protein, 20 aa, Homo sapiens
MTPEDLTAIGVTKPGHRKKI

SEQ ID NO: 39 - protein, 20 aa, Homo sapiens
LEDIGSMFDDLADQLDAMLE

SEQ ID NO: 40 - protein, 20 aa, Homo sapiens
LDDISTMFDALADQLDAMLD

SEQ ID NO: 41 - protein, 20 aa, Homo sapiens
GMPAWYVAACRANVKSGAIM

SEQ ID NO: 42 - protein, 33 aa, Xenopus borealis
GRKKRRQRRRCDLAEHTEHLKANDNLKSQEYES

SEQ ID NO: 43 - protein, 32 aa, Green anole (PTP Sigma)
GRKKRRQRRRCDHTEHLKANDNLKLSQEYESI

SEQ ID NO: 44 - protein, 35 aa, Danio rerio
GRKKRRQRRRCELAEHTELLKANDNLKLSQEYESI

SEQ ID NO: 45 - protein, 35 aa, Tilapia nilotica; identical to SEQ ID NO: 44

SEQ ID NO: 46 - protein, 35 aa, Gallus gallus
GRKKRRQRRRCELAEHTEHLKANDNLKLSQEYESI

SEQ ID NO: 47 - protein, 35 aa, Fringilla coelebs; identical to SEQ ID NO: 46

SEQ ID NO: 48 - protein, 35 aa, Ornithorhynchus anatinus
GRKKRRQRRRCELAEHTDHLKANDNLKLSQEYESI

SEQ ID NO: 49 - protein, 35 aa, Sarcophilus harrisii
GRKKRRQRRRCEMAEHTEHLKANDNLKLSQEYESI

SEQ ID NO: 50 - protein, 35 aa, Mustela putorius
GRKKRRQRRRCDMAEHTERLKANDSLKLSQEYESI

SEQ ID NO: 51 - protein, 35 aa, Galago alleni; identical to SEQ ID NO: 50

SEQ ID NO: 52 - protein, 35 aa, Callithrix argentata; identical to SEQ ID NO: 50

SEQ ID NO: 53 - protein, 35 aa, Rattus rattus
GRKKRRQRRRCDMAEHMERLKANDSLKLSQEYESI

SEQ ID NO: 54 - protein, 35 aa, Mus musculus; identical to SEQ ID NO: 53

SEQ ID NO: 55 - protein, 35 aa, Canis familiaris; identical to SEQ ID NO: 50

SEQ ID NO: 56 - protein, 35 aa, Sus barbatus; identical to SEQ ID NO: 50

SEQ ID NO: 57 - protein, 35 aa, Bos primigenius; identical to SEQ ID NO: 50

SEQ ID NO: 58 - protein, 35 aa, Ovis aries; identical to SEQ ID NO: 50

SEQ ID NO: 59 - protein, 35 aa, Orcinus orca; identical to SEQ ID NO: 50

SEQ ID NO: 60 - protein, 35 aa, Saimiri boliviensis; identical to SEQ ID NO: 50

SEQ ID NO: 61 - protein, 35 aa, Papio hamadryas; identical to SEQ ID NO: 50

SEQ ID NO: 62 - protein, 35 aa, Primate calicivirus; identical to SEQ ID NO: 50

SEQ ID NO: 63 - protein, 35 aa, Primate calicivirus; identical to SEQ ID NO: 50

SEQ ID NO: 64 - protein, 35 aa, Macaca arctoides; identical to SEQ ID NO: 50

SEQ ID NO: 65 - protein, 35 aa, Chimpanzee (PTP Sigma); identical to SEQ ID NO: 50

SEQ ID NO: 66 - protein, 35 aa, Homo sapiens; identical to SEQ ID NO: 50

SEQ ID NO: 67 - protein, 10 aa, Homo sapiens
DMAEHTERLK

SEQ ID NO: 68 - protein, 4 aa, Homo sapiens
ANDS

SEQ ID NO: 69 - protein, 10 aa, Homo sapiens
LKLSQEYESI

SEQ ID NO: 70 - protein, 25 aa, synthetic construct
  VARIANT 14: note = X is any naturally occuring amino acid or X is T or M
GRKKRRQRRRCEHXERLKANDSLKL

SEQ ID NO: 71 - protein, 31 aa, Homo sapiens
GRKKRRQRRRCMTPEDLTAIGVTKPGHRKKI

SEQ ID NO: 72 - protein, 31 aa, Homo sapiens
GRKKRRQRRRCLEDIGSMFDDLADQLDAMLE

SEQ ID NO: 73 - protein, 31 aa, Homo sapiens
GRKKRRQRRRCLDDISTMFDALADQLDAMLD

SEQ ID NO: 74 - protein, 31 aa, Homo sapiens
GRKKRRQRRRCGMPAWYVAACRANVKSGAIM

SEQ ID NO: 75 - protein, 29 aa, Homo sapiens
VSVNVLNDIGNMANLTDELDAMLEEEKRV

SEQ ID NO: 76 - protein, 25 aa, Mus musculus
STGSILEDIGSMFDDLADQLDAMLE

SEQ ID NO: 77 - protein, 25 aa, Rattus rattus
STGSILEDIGSMFDDLADQLDAMLE

SEQ ID NO: 78 - protein, 29 aa, Homo sapiens
VSVNVLNDIGNMANLTDELDAMLEEEKRV

SEQ ID NO: 79 - protein, 25 aa, Mus musculus
STKHILDDISTMFDALADQLDAMLD

SEQ ID NO: 80 - protein, 25 aa, Rattus rattus
STKHILDDISTMFDALADQLDAMLD

SEQ ID NO: 81 - protein, 30 aa, Homo sapiens
PTIARMTPEDLTAIGIKNPHHRERIKQRID

SEQ ID NO: 82 - protein, 30 aa, Mus musculus
PTISRMTPEDLTAIGVTKPGHRKKITAEIS

SEQ ID NO: 83 - protein, 30 aa, Mus musculus
PTISRMTPEDLTAIGVTKPGHRKKIASEIA

SEQ ID NO: 84 - protein, 30 aa, Rattus rattus; identical to SEQ ID NO: 82

SEQ ID NO: 85 - protein, 30 aa, Rattus rattus; identical to SEQ ID NO: 83

SEQ ID NO: 86 - protein, 30 aa, Homo sapiens; identical to SEQ ID NO: 83

SEQ ID NO: 87 - protein, 30 aa, Mus musculus
WLELWGMPAWYVAACRANVKSGAIMSALSD

SEQ ID NO: 88 - protein, 30 aa, Mus musculus
WLELWGMPAWYVAACRANVKSGAIMANLSD

SEQ ID NO: 89 - protein, 30 aa, Mus musculus; identical to SEQ ID NO: 87

SEQ ID NO: 90 - protein, 30 aa, Rattus rattus; identical to SEQ ID NO: 87

SEQ ID NO: 91 - protein, 30 aa, Rattus rattus; identical to SEQ ID NO: 87

SEQ ID NO: 92 - protein, 30 aa, Rattus rattus; identical to SEQ ID NO: 88

SEQ ID NO: 93 - protein, 30 aa, Rattus rattus; identical to SEQ ID NO: 87